European Patent Application EP 4 803 639 A1, published September 9, 2026. Title: Composition for detecting Cutibacterium acnes YM-1 strain and uses thereof. Applicant: 코스맥스 주식회사. The sequence listing filed with the application follows.

SEQUENCE LISTING (3 sequences)

SEQ ID NO: 1 - DNA, 119 bp, Cutibacterium acnes
  source 1..119: mol_type = genomic DNA
agaccagtggggtgggcgtcttcgacggtgtccggctgccagaccactaagaggcctggcagccgggcggcccagatcgactgcgagatgattccaccccggatatgagctgaggaact

SEQ ID NO: 2 - DNA, 22 bp, synthetic construct
  source 1..22: mol_type = other DNA
agaccagtggggtgggcgtctt

SEQ ID NO: 3 - DNA, 22 bp, synthetic construct
  source 1..22: mol_type = other DNA
agttcctcagctcatatccggg